European Patent Application EP 4 218 936 A1, published August 2, 2023. Title: Feeds and compositions comprising lactic acid bacteria and fatty acids. Applicant: HOUSE WELLNESS FOODS CORPORATION. The sequence listing filed with the application follows.

SEQUENCE LISTING (4 sequences)

SEQ ID NO: 1 - DNA, 24 bp, Artificial Sequence
  primer
tgtctcacctgctatttgccttac

SEQ ID NO: 2 - DNA, 29 bp, Artificial Sequence
  primer
catacacattctctctaagtttccactgt

SEQ ID NO: 3 - DNA, 20 bp, Artificial Sequence
  primer
cctctctggcaaagtccaag

SEQ ID NO: 4 - DNA, 20 bp, Artificial Sequence
  primer
catctgcccatttgatgttg